European Patent Specification EP 3 795 169 B1, published August 23, 2023. Title: Novel recombinant protein from bacteriophage having antibacterial activity to pathogenic gram-negative bacterium. Applicant: KYUNGPOOK NATIONAL UNIVERSITY INDUSTRY-ACADEMIC COOPERATION FOUNDATION. The sequence listing filed with the application follows.

SEQUENCE LISTING (2 sequences)

SEQ ID NO: 1 - protein, 170 aa, Artificial Sequence
  LysSS
MSNRNISNNGIKFTAAFEGFRGTAYRATKNEKYLTIGYGHYGADVKEGQKITEGQGLLLLHKDMAKAVAAVDAVAHPSLNQSQFDAMCDLVYNAGAGVIAASTGTGQALRKGDVATLRNKLSQFHYQNGKSLLGLRRRAAGRVALFDGMLWQQAEAIGREAKLEHHHHHH

SEQ ID NO: 2 - DNA, 486 bp, Artificial Sequence
  LysSS
atgtcaaaccgaaacattagtaacaacggcatcaaattcaccgccgcgttcgagggtttccgtggaaccgcgtacagggcgacgaagaacgagaagtacctgacaattggctacggccactacggcgcagatgtgaaagagggccagaaaattaccgagggacagggtcttctgctgctgcacaaggatatggctaaggccgtagctgcggtagacgctgtagcgcatccgtcgctcaatcagtcacagttcgatgcgatgtgcgacctggtgtataacgctggcgccggtgtgattgcggcttctaccggaacagggcaggccctgcgtaagggcgacgttgccacactgcggaataagctatctcagttccattatcagaacggcaaatcactccttggattgcgtcggcgtgccgcgggtcgtgttgcgctattcgacggtatgctgtggcaacaggcggaagccatcggccgcgaagcaaag